European Patent Specification EP 3 458 606 B1, published April 2, 2025. Title: METHODS FOR IDENTIFICATION OF SAMPLES. Applicant: DName-iT NV Cuppens, Harry. The sequence listing filed with the application follows.

SEQUENCE LISTING (20 sequences)

SEQ ID NO: 1 - DNA, 401 bp, Artificial Sequence
  barcode flanking region
aagctttgtggatgtacaagtccacaccatgtacactagacgcagcctgtacagatatccatccagtgtactcactgtcgacacggatccaatgcccgggttctgatagacgaacgacgagatgtgcagtgacttcgaggatcccagatgtgcacgtagtgcaggtagcttgaatgactactacgcctgtagcatcatcacgtagactcgtacagctacatgacggtagctagattgacgactcaagcatgctagtgtcgttactgacctgatgacacagtcgatgcgaccttaatacgactcactatagggtcaacaagaccctgcagatcccgggatccgcctcttaagctgcgcaggccaggaattgcacgtcagagcactaaggccgccaccatggc

SEQ ID NO: 2 - DNA, 401 bp, Artificial Sequence
  barcode flanking region
aagctttgtggatgtacaagtccacaccatgtacactagacgcagcctgtacagatatccatccagtgtactcactgtcgacacggatccaatgcccgggttctgatagacgaacgacgagatgtgcagtgacttcgaggatcccagatgtgcacgtagtgcaggtagcttgaatgactactacgcctgtagcatcatcacgtagactcgtacagctacatgacggtagctagattgacgactcaagcatgctagtgtcgttactgacctgatgacacagtcgatgcgaccttaaatgctgagagattagggtcaacaagaccctgcagatcccgggatccgcctcttaagctgcgcaggccaggaattgcacgtcagagcactaaggccgccaccatggc

SEQ ID NO: 3 - DNA, 401 bp, Artificial Sequence
  constant sequence
aagcttctctcgccagctatttaaagtacgagtcgggaggccttagcacgaactgatttttccagcctgagtgctgttcttgcatgtaccttctatctaacgacgtccgtaataggaagtataccaggtcgaactaacgactcctttgccgtagcgagtgtttcgccaaaagtgtctgggtctactggccaccgtccagcatttctatgcccgtaccaggacccttcgtgtaatcccccatggattttcaagaattgaggaaaagtcacgtctccaaggccctacagggccagcggatactttgaaagcgacgataatatggtcgcttatttcatccaagccccgcgctaaacatggattttgggatgctatcccgaaagtacgacttggctccaaaggcc

SEQ ID NO: 4 - DNA, 401 bp, Artificial Sequence
  barcode flanking region
aagcttaacttcagctgaagacccgttttcgatccgcggcgagcccggagtgtaaaacgatagacgtgatgcttcggtcttctcaccccttcgaggtcataacatttttgtcatgattgccgtagtgctgatagtcctgagtctaaggcattcaatacaacgtacctcaggtcaattagactgtccatgactcatcttccgaagcgcagaatgatacgcagttctcactagttgggacctgctcgacgtccggttaaggcggatttaactaagcatagggtaccgtcacctgggcaactgaaaatggcctctgtgacgcaagatgcatgttcggtcagctcgttcaaagacggtatgaaatagagtagacatcagtacatcactcggacaggagcacctat

SEQ ID NO: 5 - DNA, 401 bp, Artificial Sequence
  barcode flanking region
aagcttgcgcaactttgacgaaatgttggccaatagcatacccgaacaccgcagggttaatgcctacagctagtgttagtcgttccggtagacatctgttaaagccggaagctcgcccgactgtacgaaatcacatctaactatacaactgcgccactttgcaaatcgagtcacgacgacctgtcccttacggtgcccatttgcgctgtaatgccgatcacttcacacaaacaaggcgcttgagagctcgaacttaggcgatgagggacaagtggtacccaagctccaatagtagaatgtgtaccatagggccgcggcgagccgcctttgtatcctgaaaaaattctcatcggcagcgcagtttattatttagttggaagcattagtgaacataacagcgc

SEQ ID NO: 6 - DNA, 401 bp, Artificial Sequence
  barcode flanking region
aagcttccgtggtgggcagaagagcctagcttactctttatttaaaaacgccagtagaatttggtcgggaggatacgatccactgtccaacataaataacccgctgtagcctttacacattcacgggttaagtgtagtgcgtgttctgtgtttctggtttgaataactgttcccactgtcttgaggatcgattctggccaaaatgtatgaccctctacataggatgtacccctggggtaggacggaatcgattacgacccctgatgataatgaccaatcgtgacggtcggtgtctactgacttcgcctacatccgacgatcctggctaggcgggttgagaacatcacggtattggggatcgggatgcgcgatcgcgataatgtggacttcgcaggtagtag

SEQ ID NO: 7 - DNA, 401 bp, Artificial Sequence
  barcode flanking region
aagcttggtggagcgcaaattctatttctgagttgcggcgtcagttgccattgaagtgcccgagctgcatagtctcacggtgagtcctcttgtacgaccactagatgcaatgaagcgtgcatggagcgccactctgcaataaaagccgaaacgctctgtaaacaagattaatgtctcgtgatgctctgaaaccgtttacctaacacgaacgataagacgcaacatcttccagagatgattacccgacacgctaatgaccgttatcactccccgcacatctgagcgtactttttgaagtcccgaggattgtcacggactaaatacctcgaatatcctgaactacctttgccaatggagggaaggacagggacacgctgtcggtactttgtaggcatttgggt

SEQ ID NO: 8 - DNA, 401 bp, Artificial Sequence
  barcode flanking region
aagcttagctcgacgcacaatccaacaagtagcactgctgtctactaagcaacgtaatgatccattcagacgagtttggaatgatctgcctcacccaaagcattaggcagccccctagctttctataggagaccgaaagagcatgagagagaactccctgatgacttactgactgcgtgatggttggctccgggacgcgcaacgcaacactttgtgtggcacgtaacttgtcgcacatatgtaatagcttcaaacccgcctcgtcttctggtgtgcgctcgttcatttaatcgaatagattcctctctctactgctggtcaagggcgtattggaaataacaagcaagctcctccgagctgagctacgagtcgatccgcccatgttccctcattatcgtctg

SEQ ID NO: 9 - DNA, 401 bp, Artificial Sequence
  barcode flanking region
aagcttgacctgtagcaccgcaaataatcattgctaatacgattcaagaatcgccctcgttatttgtattcacaggtgacccttggcttctactctaacacctaaggctgatccaactcagacttaagcggcgcagccgcaaatgtaatatgttcactgagagagagacgacggctccgtaggtcgaacattcaggtagctggagagatcattgcttagcatggcgctcgcggatctgttactgcaaatggcaacagactagaaaacaggcctaatatgatctcggaattttcgcctaacacgctcctttgactggctgtgaggcctaagcgattctggcagcgctgtgacttatcaagacacgcatgtcactacttgaccggcatcgtgccactctacgc

SEQ ID NO: 10 - DNA, 401 bp, Artificial Sequence
  barcode flanking region
aagcttttctctgcaacaggcgactatcggggccgggtgccaatctttcaaaagtgtgtaaacgtgcgaccgccagatgtcatgattcaatgtcttacctcgggctatcgtcataataagtttctaccgtaaggcacgccctaaggacgttccgaataaacacgcacccccccgtcgtttcagaaatctcattaccggctgacatgcctttagatacctcagagaaatctaaccacgtgtgttacgactgacgtctcaaagagacgagctgctcctagctttcctattggagtatctgtgcctcttgtgtcgggatttagtggatcaatatgctcccctacgataggtaagatttacccgttcgtcaattagagagccgggttttattattcggtcggcag

SEQ ID NO: 11 - DNA, 400 bp, Artificial Sequence
  barcode flanking region
catcatcaccatcaccattgatctcccagctgtgacacaaataagctagcccggggcagcatggaggttaaaattgtgcatccgaccggccaggatacgtaatattaatgcgcaccgcgcactgaagaatatgatcgaggctcgctgtagcagcactcagaaaaaaaaaaaaaaaaaaaaaaaaagagtgaataacactcagatctcgggggcgtgaatgctaaacatacacagagcacgcggtgatgtataccgctatgtcggtcatgtgctacctacagaagagctaggagtggatgagcactacacggtttcgggctaagaccatactctcacacgtgtggatgactcgagacagcagtgtcagagcatgtagctctagagatgacacgatgaattc

SEQ ID NO: 12 - DNA, 400 bp, Artificial Sequence
  barcode flanking region
catcatcaccatcaccattgatctcccagctgtgacacaaataagctagcccggggcagcatggaggttaaaattgtgcatccgaccggccaggatacgtaatattaatgcgcaccgcgcactgaagaatatgatcgaggctcgctgtagcagcactcagaaccgtaataggaagtataccaaaagagtgaataacactcagatctcgggggcgtgaatgctaaacatacacagagcacgcggtgatgtataccgctatgtcggtcatgtgctacctacagaagagctaggagtggatgagcactacacggtttcgggctaagaccatactctcacacgtgtggatgactcgagacagcagtgtcagagcatgtagctctagagatgacacgatgaattc

SEQ ID NO: 13 - DNA, 400 bp, Artificial Sequence
  barcode flanking region
cctctacggctccgtatcttaagacaaatgcgttctcgtaggtttgcttctacgtgatcatccggggtggtaatccgccctcgatctcctaaggatgaaaagggttagttgggccgaatttagttgatcgataagctgacggaaatctttactagcggataagctcatcccttcctgggtcaagatgcgagctagtacggccgcgtcgctaatctcaatgaccattaactttgcgtagccatgtgtgctgctgcggagcgatactattaattgccctttcagttctggttccattgcactctgaaggatctccagtttgtcggaatatcacgtaagaacgcttggcagaaaaagtctctatgctgtaacgcctcgacgtgaaactcgacaatgtgaattc

SEQ ID NO: 14 - DNA, 400 bp, Artificial Sequence
  barcode flanking region
cgtgaggggcacggcgagggagatcacaatatactgtcgtcgtttgatttcggaacagagccaacgggttcgggtgtcttgtgtgcttcactacatgacctcggtaaccagcagatttggtccaccgggtttgtgctggatttaggacaaggcgaaatatcatgatatacacagcatcgctttgccgttacatttttggcagccaaatggatcagaggctggtggggattacaccaccttgcccttacattggctaacgttttcaacacgtgttcctaaaatgtcagtcatgtccccccacacactatagcgctgagtcgatggagatcaaatgaggaatcgaccggaaaccttggtgtcactgcctatgcgccggcaatgaacaaaccgaagtgaattc

SEQ ID NO: 15 - DNA, 400 bp, Artificial Sequence
  barcode flanking region
aagctggtagcatatggatagctggcatgttcagataattgctatctggtatccccacggatgctgatggctgatctttaaggtaaatgacattcgttgtctttacgcgccacagtgttgggccaagcagtctagtcatccagggtcatgctgagtctgcctcgtagcttaaactgttctaccattacgcggtcacgagccgtgacatctcctatttacctggcacggttgcggtggcttgtaccgctccagatattataggagtcaagtctaatgtcttatttatgcgagcgtcataggaccttgtccaataaattgaaaggatacgcccgagctgtggtagctgttagtgacggcatattgccgagggagccatcgaatgcaatgttgattcgaattc

SEQ ID NO: 16 - DNA, 400 bp, Artificial Sequence
  barcode flanking region
gtgctgttttgttcctcagttcgatacgacctaggaactgatggcgggctacccggatgatctcgatttgttctctcatgatagcaacggcgtcaagcgtcagtcttgtctcgatggagggtcgagtagatttggcttggatctttctcgtgtaaagtaaatccctgccagaggaccgagctggacggcgaagaagtttttttatctctgcacttcgaacgataagcgtcgtctccctggtcgcaaacatgggcccaaattggcttgcgattgttaaactaccggagtttttaatcgcctaaaccgcggagttaatccatgcaaccaagccagtaggatgaagaagtgcgtccagtcgatcgttagtgcctggaatttctcttatcggcatcaagaattc

SEQ ID NO: 17 - DNA, 400 bp, Artificial Sequence
  barcode flanking region
tgtccgctctctagcagaagttgtaagttttaactcagtaggctgctactgaggggattgaacgcatgttatttgggttagtggtaataaatgactgtctcaggcgccatgctagagaacaattttgctggtttgcttacatggagacactagtctggtaccgcaccactcatggaatcaagcgtggtaggcccattgtttacgtacgagccggctgcatgagggcacatagcatctggataaggcccgagagacagaggtctgccgagttttacgataccatagctgttgcgccttgcattgctatcggttttacctgtcgtctccggcagacggtttattcctcactcaattaattggctagtgcggctggttatccaacaagcgcattagtgaattc

SEQ ID NO: 18 - DNA, 400 bp, Artificial Sequence
  barcode flanking region
ccggtaacttgctcctgggacgcttaaatggcaattttaaaggaggcgaccgacccccctaacctaaggatggtacttggtgaatactatcaaccacctccgtgacggcggccaattcaatcctgtaacgcgtgtcgtaaaagttcagtttgtcgcagggtcgagttacccgtaatcctgggaacgcccccccaatccgcttcagggctatatgccacacttgaaatcggaagtatcttggcttgagtatagtctggcgtggtaccacacatctacagtgaggtgaaaggcgcttctggcaaggtacgttctgcctgacagaattattcgcattagtggatgcgtccctggagtgcgtaaagcacactcggcagatgagtgctcggagcggactgaattc

SEQ ID NO: 19 - DNA, 400 bp, Artificial Sequence
  barcode flanking region
tagatgttgtacctgacaaccttctccctgcaaagcgggtgcctaaagatgttgttacatactccaggcctcgatatggtccaatcaaaatcccatcggaccagcgttggaaagtagcacataagcgtgagacctcaggagatccgtgtataagtgaatactggcattgggggtagttactagtgccgttcaatcggggaatgactcgggacataacgtctctaatctatatgagggtaccatattcaccgtaaaagactagagtccaatttggcctttcctcttagggaagagagtacaaaccgaaaacctggcgatcacgcctgcacagcagaatcttgcctcgtttgtgtatcattgtggcagaggagcctttaagacatgcgaatagatcgaattc

SEQ ID NO: 20 - DNA, 400 bp, Artificial Sequence
  constant sequence
gattttgtcgtaaaacgatcatcatgagatcaagttcgtagaagccctgtcatatttaggagtttgatgatcggcgcgagtgtaagtagcacaccgtattccaccgtgtttacctaacgcgactgcacagtactggcaggtaacgtacaaactcatacaagggtttccacctctggcatgcttcttcggtatctcgttcgatgtcgcattaatgcgttgaggaatggggttcatctggtcagggtctgaccgtttgtaaactaggtgacgagcctgcggacctgatgtttaatctagcgccctttatggaaatctgttacgcgcagccagatgtgttgtatcgagggatgtctaggtcctacacgcgacgatgaaacgggttcgtgtcggataggaattc